European Patent Application EP 4 559 936 A1, published May 28, 2025. Title: ANTI-ADRENOMEDULIN NON-NEUTRALIZING ANTIBODY, METHOD FOR PREPARING SAME, AND USE THEREOF. Applicant: 上海济煜医药科技有限公司. Application WO PCT/CN2023/108389, filed July 20, 2023. The sequence listing filed with the application follows.

SEQUENCE LISTING (61 sequences)

SEQ ID NO: 1 - protein, 16 aa, synthetic construct
YRQSMNNFQGLRSFGC

SEQ ID NO: 2 - protein, 21 aa, synthetic construct
YRQSMNNFQGLRSFGCRFGTC

SEQ ID NO: 3 - protein, 19 aa, synthetic construct
YRQSMNQGSRSNGCRFGTC

SEQ ID NO: 4 - protein, 52 aa, synthetic construct
YRQSMNNFQGLRSFGCRFGTCTVQKLAHQIYQFTDKDKDNVAPRSKISPQGY

SEQ ID NO: 5 - protein, 50 aa, synthetic construct
YRQSMNQGSRSNGCRFGTCTFQKLAHQIYQLTDKDKDGMAPRNKISPQGY

SEQ ID NO: 6 - DNA, 20 bp, synthetic construct
  source 1..20: mol_type = other DNA
ggacagggmtccakagttcc

SEQ ID NO: 7 - DNA, 28 bp, synthetic construct
  source 1..28: mol_type = other DNA
gcacacgactgaggcacctccagatgtt

SEQ ID NO: 8 - DNA, 42 bp, synthetic construct
  source 1..42: mol_type = other DNA
aagcagtggtatcaacgcagagtcatcccccccccccccccc

SEQ ID NO: 9 - protein, 119 aa, synthetic construct
QIQLVQSGPELRKPGETVKISCKASGYAFTTFGMSWIKQAPGQGLKWMGWINTYSRVPKYTDDFKGRFAFSLEISATTAYLLINNLKNGDTATYFCARGYGGEGGLGFSGQGTTLTVSS

SEQ ID NO: 10 - protein, 112 aa, synthetic construct
DVLMTQTPFSLPVSLGDQASISCRSSQSIIDSDGNTYLEWYLQKPGQSPKLLIYKVSNRFSGVPDRFSGSGSGTDFTLRISRVEAEDLGVYYCFQGSHFPYTFAGGTKLELK

SEQ ID NO: 11 - protein, 7 aa, synthetic construct
GYAFTTF

SEQ ID NO: 12 - protein, 6 aa, synthetic construct
NTYSRV

SEQ ID NO: 13 - protein, 10 aa, synthetic construct
GYGGEGGLGF

SEQ ID NO: 14 - protein, 16 aa, synthetic construct
RSSQSIIDSDGNTYLE

SEQ ID NO: 15 - protein, 7 aa, synthetic construct
KVSNRFS

SEQ ID NO: 16 - protein, 9 aa, synthetic construct
FQGSHFPYT

SEQ ID NO: 17 - protein, 119 aa, synthetic construct
QIQLVQSGSELKKPGASVKVSCKASGYAFTTFGMSWIRQAPGQGLEWMGWINTYSRVPKYTQGFTGRFVFSLDISVTTAYLQISSLKAEDTAVYFCARGYGGEGGLGFSGQGTLVTVSS

SEQ ID NO: 18 - protein, 112 aa, synthetic construct
DVVMTQSPLSLPVTLGQPASISCRSSQSIIDSDGNTYLEWYQQRPGQSPRLLIYKVSNRFSGVPDRFSGSGSGTDFTLKISRVEAEDFGVYYCFQGSHFPYTFGQGTKLEIK

SEQ ID NO: 19 - protein, 112 aa, synthetic construct
DVLMTQSPLSLPVTLGQPASISCRSSQSIIDSDGNTYLEWYQQRPGQSPRLLIYKVSNRFSGVPDRFSGSGSGTDFTLKISRVEAEDFGVYYCFQGSHFPYTFAQGTKLEIK

SEQ ID NO: 20 - protein, 107 aa, synthetic construct [sequence omitted]

SEQ ID NO: 21 - protein, 330 aa, synthetic construct [sequence omitted]

SEQ ID NO: 22 - protein, 219 aa, synthetic construct
DVLMTQTPFSLPVSLGDQASISCRSSQSIIDSDGNTYLEWYLQKPGQSPKLLIYKVSNRFSGVPDRFSGSGSGTDFTLRISRVEAEDLGVYYCFQGSHFPYTFAGGTKLELKRTVAAPSVFIFPPSDEQLKSGTASVVCLLNNFYPREAKVQWKVDNALQSGNSQESVTEQDSKDSTYSLSSTLTLSKADYEKHKVYACEVTHQGLSSPVTKSFNRGEC

SEQ ID NO: 23 - protein, 449 aa, synthetic construct
QIQLVQSGPELRKPGETVKISCKASGYAFTTFGMSWIKQAPGQGLKWMGWINTYSRVPKYTDDFKGRFAFSLEISATTAYLLINNLKNGDTATYFCARGYGGEGGLGFSGQGTTLTVSSASTKGPSVFPLAPSSKSTSGGTAALGCLVKDYFPEPVTVSWNSGALTSGVHTFPAVLQSSGLYSLSSVVTVPSSSLGTQTYICNVNHKPSNTKVDKKVEPKSCDKTHTCPPCPAPELLGGPSVFLFPPKPKDTLMISRTPEVTCVVVDVSHEDPEVKFNWYVDGVEVHNAKTKPREEQYNSTYRVVSVLTVLHQDWLNGKEYKCKVSNKALPAPIEKTISKAKGQPREPQVYTLPPSRDELTKNQVSLTCLVKGFYPSDIAVEWESNGQPENNYKTTPPVLDSDGSFFLYSKLTVDKSRWQQGNVFSCSVMHEALHNHYTQKSLSLSPGK

SEQ ID NO: 24 - protein, 219 aa, synthetic construct
DVVMTQSPLSLPVTLGQPASISCRSSQSIIDSDGNTYLEWYQQRPGQSPRLLIYKVSNRFSGVPDRFSGSGSGTDFTLKISRVEAEDFGVYYCFQGSHFPYTFGQGTKLEIKRTVAAPSVFIFPPSDEQLKSGTASVVCLLNNFYPREAKVQWKVDNALQSGNSQESVTEQDSKDSTYSLSSTLTLSKADYEKHKVYACEVTHQGLSSPVTKSFNRGEC

SEQ ID NO: 25 - protein, 449 aa, synthetic construct
QIQLVQSGSELKKPGASVKVSCKASGYAFTTFGMSWIRQAPGQGLEWMGWINTYSRVPKYTQGFTGRFVFSLDISVTTAYLQISSLKAEDTAVYFCARGYGGEGGLGFSGQGTLVTVSSASTKGPSVFPLAPSSKSTSGGTAALGCLVKDYFPEPVTVSWNSGALTSGVHTFPAVLQSSGLYSLSSVVTVPSSSLGTQTYICNVNHKPSNTKVDKKVEPKSCDKTHTCPPCPAPELLGGPSVFLFPPKPKDTLMISRTPEVTCVVVDVSHEDPEVKFNWYVDGVEVHNAKTKPREEQYNSTYRVVSVLTVLHQDWLNGKEYKCKVSNKALPAPIEKTISKAKGQPREPQVYTLPPSRDELTKNQVSLTCLVKGFYPSDIAVEWESNGQPENNYKTTPPVLDSDGSFFLYSKLTVDKSRWQQGNVFSCSVMHEALHNHYTQKSLSLSPGK

SEQ ID NO: 26 - protein, 219 aa, synthetic construct
DVLMTQSPLSLPVTLGQPASISCRSSQSIIDSDGNTYLEWYQQRPGQSPRLLIYKVSNRFSGVPDRFSGSGSGTDFTLKISRVEAEDFGVYYCFQGSHFPYTFAQGTKLEIKRTVAAPSVFIFPPSDEQLKSGTASVVCLLNNFYPREAKVQWKVDNALQSGNSQESVTEQDSKDSTYSLSSTLTLSKADYEKHKVYACEVTHQGLSSPVTKSFNRGEC

SEQ ID NO: 27 - protein, 449 aa, synthetic construct; identical to SEQ ID NO: 25

SEQ ID NO: 28 - protein, 119 aa, synthetic construct
QVQLVQSGAEVKKPGASVKVSCKASGYTFTSYGISWVRQAPGQGLEWMGWISAYNGNTNYAQKLQGRVTMTRDTSTSTAYMELRSLRSDDTAVYYCAREGRSGGSFDIWGQGTMVTVSS

SEQ ID NO: 29 - protein, 119 aa, synthetic construct
QVQLVQSGAEVKKPGASVKVSCKASGYTFTSYGISWVRQAPGQGLEWMGWISAYQGNTNYAQKLQGRVTMTRDTSTSTAYMELRSLRSDDTAVYYCAREGRSGGSFDIWGQGTMVTVSS

SEQ ID NO: 30 - protein, 119 aa, synthetic construct
QVQLVQSGAEVKKPGASVKVSCKASGYTFTSYGISWVRQAPGQGLEWMGWISAYQGNTNYAQKLQGRVTMTRDTSTSTAYMELRSLRSDDTAVYYCAREGRWGGSFNIWGQGTMVTVSS

SEQ ID NO: 31 - protein, 119 aa, synthetic construct
QVQLVQSGAEVKKPGASVKVSCKASGYTFTQYGIAWVRQAPGQGLEWMGWISAYQGNTNYAQKLQGRVTMTRDTSTSTAYMELRSLRSDDTAVYYCAREGRWGGSFNIWGQGTMVTVSS

SEQ ID NO: 32 - protein, 119 aa, synthetic construct
QVQLVQSGAEVKKPGASVKVSCKASGYTFTSYGISWVRQAPGQGLEWMGWISPYSGNTNYAQKLQGRVTMTRDTSTSTAYMELRSLRSDDTAVYYCAREGRWGGSFNIWGQGTMVTVSS

SEQ ID NO: 33 - protein, 119 aa, synthetic construct
QVQLVQSGAEVKKPGASVKVSCKASGYTFTHYGIAWVRQAPGQGLEWMGWISAYQGNTNYAQKLQGRVTMTRDTSTSTAYMELRSLRSDDTAVYYCAREGRWGGSFNIWGQGTMVTVSS

SEQ ID NO: 34 - protein, 119 aa, synthetic construct
QVQLVQSGAEVKKPGASVKVSCKASGYTFTSYGISWVRQAPGQGLEWMGWISPYTGKTNYAQKLQGRVTMTRDTSTSTAYMELRSLRSDDTAVYYCAREGRWGGSFNIWGQGTMVTVSS

SEQ ID NO: 35 - protein, 107 aa, synthetic construct
DIQMTQSPSSLSASVGDRVTITCRASQGISSYLAWYQQKPGKAPKLLIYDASNLETGVPSRFSGSGSGTDFTFTISSLQPEDIATYYCQQYDNLPLTFGGGTKVEIK

SEQ ID NO: 36 - protein, 107 aa, synthetic construct
DIQMTQSPSSLSASVGDRVTITCRASEGISEYLAWYQQKPGKAPKLLIYDASNLETGVPSRFSGSGSGTDFTFTISSLQPEDIATYYCQQYDNLPLTFGGGTKVEIK

SEQ ID NO: 37 - protein, 107 aa, synthetic construct
DIQMTQSPSSLSASVGDRVTITCRAAEGIGSYLAWYQQKPGKAPKLLIYDASNLETGVPSRFSGSGSGTDFTFTISSLQPEDIATYYCQQYDNLPLTFGGGTKVEIK

SEQ ID NO: 38 - protein, 107 aa, synthetic construct
DIQMTQSPSSLSASVGDRVTITCRASQGISSYLAWYQQKPGKAPKLLIYDVSILDAGVPSRFSGSGSGTDFTFTISSLQPEDIATYYCQQYDNLPLTFGGGTKVEIK

SEQ ID NO: 39 - protein, 107 aa, synthetic construct
DIQMTQSPSSLSASVGDRVTITCRASQGISSYLAWYQQKPGKAPKLLIYDASNVDTGVPSRFSGSGSGTDFTFTISSLQPEDIATYYCQQYDNLPLTFGGGTKVEIK

SEQ ID NO: 40 - protein, 107 aa, synthetic construct
DIQMTQSPSSLSASVGDRVTITCRASQGISSYLAWYQQKPGKAPKLLIYDTSDLDTGVPSRFSGSGSGTDFTFTISSLQPEDIATYYCQQYDNLPLTFGGGTKVEIK

SEQ ID NO: 41 - protein, 107 aa, synthetic construct
DIQMTQSPSSLSASVGDRVTITCRASQGISSYLAWYQQKPGKAPKLLIYDASNLETGVPSRFSGSGSGTDFTFTISSLQPEDIATYYCQQYDDLDLTFGGGTKVEIK

SEQ ID NO: 42 - protein, 107 aa, synthetic construct
DIQMTQSPSSLSASVGDRVTITCRASQGISSYLAWYQQKPGKAPKLLIYDASNLETGVPSRFSGSGSGTDFTFTISSLQPEDIATYYCQQYDDLPLSFGGGTKVEIK

SEQ ID NO: 43 - protein, 7 aa, synthetic construct
GYTFTSY

SEQ ID NO: 44 - protein, 6 aa, synthetic construct
SAYNGN

SEQ ID NO: 45 - protein, 10 aa, synthetic construct
EGRSGGSFDI

SEQ ID NO: 46 - protein, 11 aa, synthetic construct
RASQGISSYLA

SEQ ID NO: 47 - protein, 7 aa, synthetic construct
DASNLET

SEQ ID NO: 48 - protein, 9 aa, synthetic construct
QQYDNLPLT

SEQ ID NO: 49 - protein, 6 aa, synthetic construct
SAYQGN

SEQ ID NO: 50 - protein, 10 aa, synthetic construct
EGRWGGSFNI

SEQ ID NO: 51 - protein, 7 aa, synthetic construct
GYTFTQY

SEQ ID NO: 52 - protein, 11 aa, synthetic construct
RASEGISEYLA

SEQ ID NO: 53 - protein, 11 aa, synthetic construct
RAAEGIGSYLA

SEQ ID NO: 54 - protein, 6 aa, synthetic construct
SPYSGN

SEQ ID NO: 55 - protein, 7 aa, synthetic construct
GYTFTHY

SEQ ID NO: 56 - protein, 7 aa, synthetic construct
DVSILDA

SEQ ID NO: 57 - protein, 7 aa, synthetic construct
DASNVDT

SEQ ID NO: 58 - protein, 6 aa, synthetic construct
SPYTGK

SEQ ID NO: 59 - protein, 7 aa, synthetic construct
DTSDLDT

SEQ ID NO: 60 - protein, 9 aa, synthetic construct
QQYDDLDLT

SEQ ID NO: 61 - protein, 9 aa, synthetic construct
QQYDDLPLS